European Patent Application EP 4 696 310 A2, published February 18, 2026. Title: METHODS AND COMPOSITIONS FOR MODULATION OF TAU PROTEINS. Applicant: SANGAMO THERAPEUTICS, INC. The sequence listing filed with the application follows.

SEQUENCE LISTING (13 sequences)

SEQ ID NO: 1 - DNA, 28 bp, unidentified
  source 1..28: mol_type = unassigned DNA; note = Description of Unknown: Human or mouse oligonucleotide
tggtgctggagctggtgggtggcggaga

SEQ ID NO: 2 - DNA, 28 bp, Mus sp.
  source 1..28: mol_type = genomic DNA
cggcagaaggtgggcggtggcggcggcg

SEQ ID NO: 3 - protein, 7 aa, synthetic construct
  source 1..7: note = Description of Artificial Sequence: Synthetic peptide
LRHHLTR

SEQ ID NO: 4 - protein, 7 aa, synthetic construct
  source 1..7: note = Description of Artificial Sequence: Synthetic peptide
RRFTLSK

SEQ ID NO: 5 - protein, 7 aa, synthetic construct
  source 1..7: note = Description of Artificial Sequence: Synthetic peptide
RSDVLSE

SEQ ID NO: 6 - protein, 7 aa, synthetic construct
  source 1..7: note = Description of Artificial Sequence: Synthetic peptide
KHSTRRV

SEQ ID NO: 7 - protein, 7 aa, synthetic construct
  source 1..7: note = Description of Artificial Sequence: Synthetic peptide
RLYTLHK

SEQ ID NO: 8 - protein, 7 aa, synthetic construct
  source 1..7: note = Description of Artificial Sequence: Synthetic peptide
DRSHLTR

SEQ ID NO: 9 - protein, 7 aa, synthetic construct
  source 1..7: note = Description of Artificial Sequence: Synthetic peptide
LKQHLTR

SEQ ID NO: 10 - protein, 7 aa, synthetic construct
  source 1..7: note = Description of Artificial Sequence: Synthetic peptide
RSAHLSR

SEQ ID NO: 11 - protein, 7 aa, synthetic construct
  source 1..7: note = Description of Artificial Sequence: Synthetic peptide
TSGHLSR

SEQ ID NO: 12 - protein, 7 aa, synthetic construct
  source 1..7: note = Description of Artificial Sequence: Synthetic peptide
QSGNLAR

SEQ ID NO: 13 - protein, 7 aa, synthetic construct
  source 1..7: note = Description of Artificial Sequence: Synthetic peptide
QSGDLTR